European Patent Specification EP 4 262 745 B1, published January 29, 2025. Title: Pharmaceutical composition of GLP-1/GLP-2 dual agonists. Applicant: Zealand Pharma A/S. The sequence listing filed with the application follows.

SEQUENCE LISTING (3 sequences)

SEQ ID NO: 1 - protein, 33 aa, Artificial Sequence
  GLP-1/GLP-2 dual agonist peptide
  MOD_RES (2)..(2): Aib
  MOD_RES (16)..(16): Xaa is Lys or D-Lys in which an albumin binding moiety [K([17-carboxy-heptadecanoyl]-isoGlu)] is conjugated to the GLP-1/GLP-2 dual agonist
HXEGSFTSELATILDXQAARDFIAWLIQHKITD

SEQ ID NO: 2 - protein, 33 aa, Artificial Sequence
  GLP-1/GLP-2 dual agonist peptide (Formula A)
  MOD_RES (2)..(2): Aib
  MISC_FEATURE (5)..(5): Xaa is Thr or Ser
  MISC_FEATURE (7)..(7): Xaa is Thr or Ser
  MISC_FEATURE (16)..(16): Xaa is Lys or D-Lys in which an albumin binding moiety [K([17-carboxy-heptadecanoyl]-isoGlu)] is conjugated to the GLP-1/GLP-2 dual agonist
  MISC_FEATURE (28)..(28): Xaa is Gln, Glu, Ala, His, Tyr, Leu, Lys, Arg or Ser
HXEGXFXSELATILDXQAARDFIAWLIXHKITD

SEQ ID NO: 3 - protein, 33 aa, Artificial Sequence
  GLP-1/GLP-2 dual agonist peptide (Formula B)
  MOD_RES (2)..(2): Aib
  MISC_FEATURE (5)..(5): Xaa is Thr or Ser
  MISC_FEATURE (16)..(16): Xaa is Lys or D-Lys in which an albumin binding moiety [K([17-carboxy-heptadecanoyl]-isoGlu)] is conjugated to the GLP-1/GLP-2 dual agonist
  MISC_FEATURE (28)..(28): Xaa is Gln, Glu, Ala, His, Tyr, Leu, Lys, Arg or Ser
HXEGXFTSELATILDXQAARDFIAWLIXHKITD